European Patent Specification EP 3 571 216 B1, published May 27, 2026. Title: APOC-II MIMETIC PEPTIDES. Applicant: THE UNITED STATES OF AMERICA, AS REPRESENTED BY THE SECRETARY, DEPARTMENT OF HEALTH AND HUMAN SERVICES CORVIDIA THERAPEUTICS, INC. Application PCT/US2018/014532. The sequence listing filed with the application follows.

SEQUENCE LISTING (73 sequences)

SEQ ID NO: 1 - protein, 79 aa, Homo sapiens
TQQPQQDEMPSPTFLTQVKESLSSYWESAKTAAQNLYEKTYLPAVDEKLRDLYSKSTAAMSTYTGIFTDQVLSVLKGEE

SEQ ID NO: 2 - protein, 40 aa, Homo sapiens
TYLPAVDEKLRDLYSKSTAAMSTYTGIFTDQVLSVLKGEE

SEQ ID NO: 3 - protein, 22 aa, Homo sapiens
QVKESLSSYWESAKTAAQNLYE

SEQ ID NO: 4 - protein, 13 aa, Homo sapiens
VDEKLRDLYSKST

SEQ ID NO: 5 - protein, 11 aa, Homo sapiens
GIFTDQVLSVL

SEQ ID NO: 6 - protein, 40 aa, Artificial Sequence
  Description of Artificial Sequence: Synthetic polypeptide
  MOD_RES (21)..(21): Norleucine
DYLKEVFEKLRDLYEKFTAALSTYTGIFTDQVLSVLKGEE

SEQ ID NO: 7 - protein, 40 aa, Artificial Sequence
  Description of Artificial Sequence: Synthetic polypeptide
DYLKEVFEKLRDLYEKFTAAVSTYTGIFTDQVLSVLKGEE

SEQ ID NO: 8 - protein, 40 aa, Artificial Sequence; identical to SEQ ID NO: 6
  Description of Artificial Sequence: Synthetic polypeptide

SEQ ID NO: 9 - protein, 40 aa, Artificial Sequence
  Description of Artificial Sequence: Synthetic polypeptide
DYLKEVFEKLRDLYEKFTPAVSTYTGIFTDQVLSVLKGEE

SEQ ID NO: 10 - protein, 40 aa, Artificial Sequence
  Description of Artificial Sequence: Synthetic polypeptide
DYLKEVFEKLRDLYEKFTPALSTYTGIFTDQVLSVLKGEE

SEQ ID NO: 11 - protein, 40 aa, Artificial Sequence
  Description of Artificial Sequence: Synthetic polypeptide
DYLKEVFEKLRDLYEKFTPAMSTYTGIFTDQVLSVLKGEE

SEQ ID NO: 12 - protein, 40 aa, Artificial Sequence
  Description of Artificial Sequence: Synthetic polypeptide
DYLREVFERLRDLYERKTPAMSTYTGIFTDQVLSVLRGEE

SEQ ID NO: 13 - protein, 40 aa, Artificial Sequence; identical to SEQ ID NO: 6
  Description of Artificial Sequence: Synthetic polypeptide
  MOD_RES (21)..(21): Norleucine

SEQ ID NO: 14 - protein, 40 aa, Artificial Sequence
  Description of Artificial Sequence: Synthetic polypeptide
  MOD_RES (21)..(21): Norleucine
DYLKEVFEKLRDLYEKKTPALSTYTGIFTDQVLSVLKGEE

SEQ ID NO: 15 - protein, 40 aa, Artificial Sequence
  Description of Artificial Sequence: Synthetic polypeptide
  MOD_RES (21)..(21): Norleucine
DYLKEVFEKLRDLYEKKTAALSTYTGIFTDQVLSVLKGEE

SEQ ID NO: 16 - protein, 40 aa, Artificial Sequence
  Description of Artificial Sequence: Synthetic polypeptide
  MOD_RES (21)..(21): Norleucine
DYLKAVFEKLRDLYSKFTAALSTYTGIFTDQVLSVLKGEE

SEQ ID NO: 17 - protein, 40 aa, Artificial Sequence
  Description of Artificial Sequence: Synthetic polypeptide
  MOD_RES (21)..(21): Norleucine
DYLKAVFEKLRDLYEKFTAALSTYTGIFTDQVLSVLKGEE

SEQ ID NO: 18 - protein, 40 aa, Artificial Sequence
  Description of Artificial Sequence: Synthetic polypeptide
  MOD_RES (21)..(21): Norleucine
DYLKAVFEKLRDLYSKFFAALSTYTGIFTDQVLSVLKGEE

SEQ ID NO: 19 - protein, 40 aa, Artificial Sequence
  Description of Artificial Sequence: Synthetic polypeptide
  MOD_RES (21)..(21): Norleucine
DYLKAVFEKLRDLYSKFTAALSTSTGIFTDQVLSVLKGEE

SEQ ID NO: 20 - protein, 40 aa, Artificial Sequence
  Description of Artificial Sequence: Synthetic polypeptide
  MOD_RES (21)..(21): Norleucine
DYLKAVFEKLRDLYSKFTAALSTYTGIFTDRVLSVLKGEE

SEQ ID NO: 21 - protein, 40 aa, Artificial Sequence
  Description of Artificial Sequence: Synthetic polypeptide
  MOD_RES (21)..(21): Norleucine
DYLKAVFEKLRDLYSKFTAALSTYTGIFTDKVLSVLKGEE

SEQ ID NO: 22 - protein, 31 aa, Artificial Sequence
  Description of Artificial Sequence: Synthetic polypeptide
  MOD_RES (12)..(12): Norleucine
KRDLYEKKFAALSTYTGIFTDQVLSVLKGEE

SEQ ID NO: 23 - protein, 40 aa, Artificial Sequence; identical to SEQ ID NO: 16
  Description of Artificial Sequence: Synthetic polypeptide
  MOD_RES (21)..(21): Norleucine

SEQ ID NO: 24 - protein, 40 aa, Artificial Sequence
  Description of Artificial Sequence: Synthetic polypeptide
  MOD_RES (21)..(21): Norleucine
DYLKAVFEKKRDLYSKFTAALSTYTGIFTDQVLSVLKGEE

SEQ ID NO: 25 - protein, 40 aa, Artificial Sequence
  Description of Artificial Sequence: Synthetic polypeptide
DYLKAVFEKLRDLYSKFTPAMSTYTGIFTDQVLSVLKGEE

SEQ ID NO: 26 - protein, 40 aa, Artificial Sequence
  Description of Artificial Sequence: Synthetic polypeptide
DYLKAVFEKLRDLYEKFTPAMSTYTGIFTDQVLSVLKGEE

SEQ ID NO: 27 - protein, 40 aa, Artificial Sequence
  Description of Artificial Sequence: Synthetic polypeptide
DYLKAVFEKLRDLYKKFTPAMSTYTGIFTDQVLSVLKGEE

SEQ ID NO: 28 - protein, 40 aa, Artificial Sequence
  Description of Artificial Sequence: Synthetic polypeptide
DYLKAVFEKLKDLYSKFTPAMSTYTGIFTDQVLSVLKGEE

SEQ ID NO: 29 - protein, 40 aa, Artificial Sequence
  Description of Artificial Sequence: Synthetic polypeptide
DWLKAVFEKLRDLYSKFTPAMSTYTGIFTDQVLSVLKGEE

SEQ ID NO: 30 - protein, 40 aa, Artificial Sequence
  Description of Artificial Sequence: Synthetic polypeptide
DYLKAVFEKLRDLYSKFFPAMSTYTGIFTDQVLSVLKGEE

SEQ ID NO: 31 - protein, 40 aa, Artificial Sequence
  Description of Artificial Sequence: Synthetic polypeptide
DYLKAFYEKLRDLLSKAFPAMSTYTGIFTDQVLSVLKGEE

SEQ ID NO: 32 - protein, 40 aa, Artificial Sequence
  Description of Artificial Sequence: Synthetic polypeptide
DYLKAVKEKLRDLYSKFTPAMSTYTGIFTDQVLSVLKGEE

SEQ ID NO: 33 - protein, 40 aa, Artificial Sequence
  Description of Artificial Sequence: Synthetic polypeptide
DYLKAVFEKKRDLYSKFTPAMSTYTGIFTDQVLSVLKGEE

SEQ ID NO: 34 - protein, 40 aa, Artificial Sequence
  Description of Artificial Sequence: Synthetic polypeptide
DYLKAVFEKLRDLYSKKTPAMSTYTGIFTDQVLSVLKGEE

SEQ ID NO: 35 - protein, 40 aa, Artificial Sequence
  Description of Artificial Sequence: Synthetic polypeptide
DYLKAVFEKLRDLYSKFTAAKSTYTGIFTDQVLSVLKGEE

SEQ ID NO: 36 - protein, 37 aa, Artificial Sequence
  Description of Artificial Sequence: Synthetic polypeptide
KAVFEKLRDLYSKFTAAKSTYTGIFTDQVLSVLKGEE

SEQ ID NO: 37 - protein, 36 aa, Artificial Sequence
  Description of Artificial Sequence: Synthetic polypeptide
DVFEKLRDLYSKFTAAKSTYTGIFTDQVLSVLKGEE

SEQ ID NO: 38 - protein, 33 aa, Artificial Sequence
  Description of Artificial Sequence: Synthetic polypeptide
EKLRDLYSKFTAAKSTYTGIFTDQVLSVLKGEE

SEQ ID NO: 39 - protein, 30 aa, Artificial Sequence
  Description of Artificial Sequence: Synthetic polypeptide
RDLYSKFTAAKSTYTGIFTDQVLSVLKGEE

SEQ ID NO: 40 - protein, 29 aa, Artificial Sequence
  Description of Artificial Sequence: Synthetic peptide
DLYSKFTAAKSTYTGIFTDQVLSVLKGEE

SEQ ID NO: 41 - protein, 26 aa, Artificial Sequence
  Description of Artificial Sequence: Synthetic peptide
DKFTAAKSTYTGIFTDQVLSVLKGEE

SEQ ID NO: 42 - protein, 40 aa, Artificial Sequence
  Description of Artificial Sequence: Synthetic polypeptide
  MOD_RES (21)..(21): Norleucine
DYLKEVFEKLRDLYSKFTAALSTYTGIFTDQVLSVLKGEE

SEQ ID NO: 43 - protein, 40 aa, Artificial Sequence
  Description of Artificial Sequence: Synthetic polypeptide
DWLKAVFEKLRDLYEKFTPAMSTYTGIFTDQVLSVLKGEE

SEQ ID NO: 44 - protein, 40 aa, Artificial Sequence
  Description of Artificial Sequence: Synthetic polypeptide
DYLKAVFEKLRDLYEKFFPAMSTYTGIFTDQVLSVLKGEE

SEQ ID NO: 45 - protein, 40 aa, Artificial Sequence
  Description of Artificial Sequence: Synthetic polypeptide
DWLKAVFEKLRDLYEKFFPAMSTYTGIFTDQVLSVLKGEE

SEQ ID NO: 46 - protein, 40 aa, Artificial Sequence
  Description of Artificial Sequence: Synthetic polypeptide
  MOD_RES (21)..(21): Norleucine
DWLKAVFEKLRDLYEKFTPALSTYTGIFTDQVLSVLKGEE

SEQ ID NO: 47 - protein, 40 aa, Artificial Sequence
  Description of Artificial Sequence: Synthetic polypeptide
  MOD_RES (21)..(21): Norleucine
DYLKAVFEKLRDLYEKFFPALSTYTGIFTDQVLSVLKGEE

SEQ ID NO: 48 - protein, 40 aa, Artificial Sequence
  Description of Artificial Sequence: Synthetic polypeptide
  MOD_RES (21)..(21): Norleucine
DWLKAVFEKLRDLYEKFFPALSTYTGIFTDQVLSVLKGEE

SEQ ID NO: 49 - protein, 21 aa, Artificial Sequence
  Description of Artificial Sequence: Synthetic peptide
AMSTYTGIFTDQVLSVLKGEE

SEQ ID NO: 50 - protein, 21 aa, Artificial Sequence
  Description of Artificial Sequence: Synthetic peptide
AMSTYTGIFTDQVLSVLKGEE

SEQ ID NO: 51 - protein, 21 aa, Artificial Sequence
  Description of Artificial Sequence: Synthetic peptide
AKSTYTGIFTDQVLSVLKGEE

SEQ ID NO: 52 - protein, 21 aa, Artificial Sequence
  Description of Artificial Sequence: Synthetic peptide
AMSTYTGIFTDQVLSVLKGEE

SEQ ID NO: 53 - protein, 40 aa, Artificial Sequence
  Description of Artificial Sequence: Synthetic polypeptide
DYLKEVFEKLRDLYEKFFPAVSTYTGIFTDQVLSVLKGEE

SEQ ID NO: 54 - protein, 40 aa, Artificial Sequence
  Description of Artificial Sequence: Synthetic polypeptide
  MOD_RES (7)..(7): Aib
  MOD_RES (17)..(17): Aib
DYLKEVXEKLRDLYEKXFPAVSTYTGIFTDQVLSVLKGEE

SEQ ID NO: 55 - protein, 40 aa, Artificial Sequence
  Description of Artificial Sequence: Synthetic polypeptide
DKVKEFLSEYWEKAKEFAPAVSTYTGIFTDQVLSVLKGEE

SEQ ID NO: 56 - protein, 40 aa, Homo sapiens
DWLKAFYDKVAEKLKEAFPAMSTYTGIFTDQVLSVLKGEE

SEQ ID NO: 57 - protein, 19 aa, Homo sapiens
TYLPAVDEKLRDLYSKSTA

SEQ ID NO: 58 - protein, 19 aa, Pan troglodytes
TYLPAVDEKLRDLYSKSTA

SEQ ID NO: 59 - protein, 19 aa, Macaca fascicularis
TYLPAVDEKLRDLYSKSTA

SEQ ID NO: 60 - protein, 19 aa, Macaca mulatta
TYLPAVDEKLRDLYSKSTA

SEQ ID NO: 61 - protein, 19 aa, Papio hamadryas
TYLPAVDEKLRDLYSKSTA

SEQ ID NO: 62 - protein, 19 aa, Callithrix jacchus
TYLHTVDEKLRDMYSKSTA

SEQ ID NO: 63 - protein, 19 aa, Mus musculus
TYPISMDEKLRDMYSKSSA

SEQ ID NO: 64 - protein, 19 aa, Rattus norvegicus
TYLTSVDEKLRDMYSKSSA

SEQ ID NO: 65 - protein, 19 aa, Canis lupus familiaris
AYPTTMDEKIRDIYSKSTA

SEQ ID NO: 66 - protein, 19 aa, Bos taurus
TYLPAVDEKIRDIYSKSTA

SEQ ID NO: 67 - protein, 19 aa, Sus scrofa
TYLPTVDEKIRDMYSKSTA

SEQ ID NO: 68 - protein, 19 aa, Cavia porcellus
TYLPAVDETIRDIYSKGSA

SEQ ID NO: 69 - protein, 18 aa, Homo sapiens
TYLPAVDEKLRDLYSKST

SEQ ID NO: 70 - protein, 18 aa, Artificial Sequence
  Description of Artificial Sequence: Synthetic peptide
DYLKAVFEKLRDLYSKFT

SEQ ID NO: 71 - protein, 18 aa, Artificial Sequence
  Description of Artificial Sequence: Synthetic peptide
DYLKEVFEKLRDLYSKFT

SEQ ID NO: 72 - protein, 18 aa, Artificial Sequence
  Description of Artificial Sequence: Synthetic peptide
DYLKEVFEKLRDLYEKFT

SEQ ID NO: 73 - protein, 18 aa, Artificial Sequence
  Description of Artificial Sequence: Synthetic peptide
DYLDAVWEKLRDLYSKFT